European Patent Specification EP 3 521 414 B1, published May 6, 2026. Title: Xylaria grammica EL 000614 strain having nematocidal activity against root knot nematode and uses thereof. Applicant: INDUSTRY FOUNDATION OF CHONNAM NATIONAL UNIVERSITY National Institute of Biological Resources. The sequence listing filed with the application follows.

SEQUENCE LISTING (6 sequences)

SEQ ID NO: 1 - DNA, 582 bp, Xylaria grammica EL 000590 ITS region sequence
gtaacaaggtctccgttggtgaaccagcggagggatcattaaagagttattacaactcccaaacccatgtgaacttaccttctgttgcctcggcaggtcgcgacctaccctgtgaggccctaccctgtagggccctacctggtagtcgcgggttacgcctgccggtggcccatgaaactctgtttattcttgttattctgaatctataactaaataagttaaaactttcaacaacggatctcttggttctggcatcgatgaagaacgcagcgaaatgcgataagtaatgtgaattgcagaattcagtgaatcatcgaatctttgaacgcacattgcgcccattagtattctagtgggcatgcctgttcgagcgtcatttcaacccttaagcccctgttgcttagcgttgggagcctacagccttctgtagctccccaaagttagtggcggagtcggtttacactctagacgtagtaaattttatctcgtctgcagttaggccggtccctcgccgtaaaaccccccaatttttaaaggttgacctcggatcaggtaggaatacccgctgaacttaagcatatc

SEQ ID NO: 2 - DNA, 581 bp, Xylaria grammica EL 000603 ITS region sequence
gtaacaaggtctccgttggtgaaccagcggagggatcattaaagagttattacaactcccaaacccatgtgaacttaccttctgttgcctcggcaggtcgcgacctaccctgtgaggccctaccctgtagggccctacctggtagtcgcgggtacgcctgccggtggcccatgaaactctgtttattcttgttattctgaatctataactaaataagttaaaactttcaacaacggatctcttggttctggcatcgatgaagaacgcagcgaaatgcgataagtaatgtgaattgcagaattcagtgaatcatcgaatctttgaacgcacattgcgcccattagtattctagtgggcatgcctgttcgagcgtcatttcaacccttaagcctctgttgcttagcgttgggagcctacagccttctgtagctccccaaagttagtggcggagtcggtttacactctagacgtagtaaattttatctcgtctgcagttaggccggtccctcgccgtaaaaccccctaatttttaaaggttgacctcggatcaggtaggaatacccgctgaacttaagcatatc

SEQ ID NO: 3 - DNA, 581 bp, Xylaria grammica EL 000614 ITS region sequence
gtaacaaggtctccgttggtgaaccagcggagggatcattaaagagttattacaactcccaaacccatgtgaacttaccttctgttgcctcggcaggtcgcgacctaccctgtgaggccctaccctgtagggccctacctggtagtcgcgggtacgcctgccggtggcccatgaaactctgtttattcttgttattctgaatctataactaaataagttaaaactttcaacaacggatctcttggttctggcatcgatgaagaacgcagcgaaatgcgataagtaatgtgaattgcagaattcagtgaatcatcgaatctttgaacgcacattgcgcccattagtattctagtgggcatgcctgttcgagcgtcatttcaacccttaagcctctgttgcttagcgttgggagcctacagccttctgtagctccccaaagttagtggcggagtcggtttacactctagacgtagtaaattttatctcgtctgcagttaggccggtccctcgccgtaaaaccccccaatttttaaaggttgacctcggatcaggtaggaatacccgctgaacttaagcatatc

SEQ ID NO: 4 - DNA, 582 bp, Xylaria grammica EL 000682 ITS region sequence; identical to SEQ ID NO: 1

SEQ ID NO: 5 - DNA, 19 bp, Artificial Sequence
  primer
tccgtaggtgaacctgcgg

SEQ ID NO: 6 - DNA, 20 bp, Artificial Sequence
  primer
tcctccgcttattgatatgc